European Patent Specification EP 3 914 249 B1, published May 1, 2024. Title: Selective Glucocorticoid Receptor Modifiers for treating impaired skin wound healing. Applicant: Akribes Biomedical GmbH. The sequence listing filed with the application follows.

SEQUENCE LISTING (4 sequences)

SEQ ID NO: 1 - DNA, 25 bp, Artificial Sequence
  EF1a probe
aagtgctaacatgccttggttcaag

SEQ ID NO: 2 - DNA, 25 bp, Artificial Sequence
  Collagen 1a probe
aagacgaagacatcccaccaatcac

SEQ ID NO: 3 - DNA, 25 bp, Artificial Sequence
  Collagen 3a probe
gaactcaagagtggagaatactggg

SEQ ID NO: 4 - DNA, 25 bp, Artificial Sequence
  IL1ß probe
cagatgaagtgctccttccaggacc